European Patent Application EP 4 275 698 A2, published November 15, 2023. Title: ANTI-TIGIT ANTIBODIES AND METHODS OF USE THEREOF. Applicant: AGENUS INC. Application EP. The sequence listing filed with the application follows.

SEQUENCE LISTING (70 sequences)

SEQ ID NO: 1 - protein, 5 aa, synthetic construct
  REGION 1..5: note = Description of Artificial Sequence: Synthetic peptide
SYGIS

SEQ ID NO: 2 - protein, 7 aa, synthetic construct
  REGION 1..7: note = Description of Artificial Sequence: Synthetic peptide
GYTFASY

SEQ ID NO: 3 - protein, 17 aa, synthetic construct
  REGION 1..17: note = Description of Artificial Sequence: Synthetic peptide
GITPFFNRVDVAEKFQG

SEQ ID NO: 4 - protein, 6 aa, synthetic construct
  REGION 1..6: note = Description of Artificial Sequence: Synthetic peptide
TPFFNR

SEQ ID NO: 5 - protein, 13 aa, synthetic construct
  REGION 1..13: note = Description of Artificial Sequence: Synthetic peptide
DLRRGGVGDAFDI

SEQ ID NO: 6 - protein, 14 aa, synthetic construct
  REGION 1..14: note = Description of Artificial Sequence: Synthetic peptide
TGTSSDVGSHNYVS

SEQ ID NO: 7 - protein, 7 aa, synthetic construct
  REGION 1..7: note = Description of Artificial Sequence: Synthetic peptide
EVSYRPS

SEQ ID NO: 8 - protein, 10 aa, synthetic construct
  REGION 1..10: note = Description of Artificial Sequence: Synthetic peptide
SSYTPSSATV

SEQ ID NO: 9 - protein, 122 aa, synthetic construct
  REGION 1..122: note = Description of Artificial Sequence: Synthetic polypeptide
  VARIANT 1: note = /replace="pyro-Glu"
  SITE 1: note = MISC_FEATURE - /note="Variant residues given in the sequence have no preference with respect to those in the annotations for variant positions"
EVQLVQSGAEVEKPGASVKVSCKASGYTFASYGISWVRQAPGQGLEWMGGITPFFNRVDVAEKFQGRVTITADTSTNTVYIELSSLTSEDTAVYYCARDLRRGGVGDAFDIWGRGTLVTVSS

SEQ ID NO: 10 - protein, 110 aa, synthetic construct
  REGION 1..110: note = Description of Artificial Sequence: Synthetic polypeptide
  VARIANT 1: note = /replace="pyro-Glu"
  SITE 1: note = MISC_FEATURE - /note="Variant residues given in the sequence have no preference with respect to those in the annotations for variant positions"
ESALTQPRSVSGSPGQSVTISCTGTSSDVGSHNYVSWYQQHPGKAPQLMIYEVSYRPSEISNRFSGSKSGNTASLTISGLQPEDEADYYCSSYTPSSATVFGAGTKLTVL

SEQ ID NO: 11 - protein, 451 aa, synthetic construct
  REGION 1..451: note = Description of Artificial Sequence: Synthetic polypeptide
  VARIANT 1: note = /replace="pyro-Glu"
  SITE 1: note = MISC_FEATURE - /note="Variant residues given in the sequence have no preference with respect to those in the annotations for variant positions"
EVQLVQSGAEVEKPGASVKVSCKASGYTFASYGISWVRQAPGQGLEWMGGITPFFNRVDVAEKFQGRVTITADTSTNTVYIELSSLTSEDTAVYYCARDLRRGGVGDAFDIWGRGTLVTVSSASTKGPSVFPLAPSSKSTSGGTAALGCLVKDYFPEPVTVSWNSGALTSGVHTFPAVLQSSGLYSLSSVVTVPSSSLGTQTYICNVNHKPSNTKVDKRVEPKSCDKTHTCPPCPAPELLGGPSVFLFPPKPKDTLMISRTPEVTCVVVDVSHEDPEVKFNWYVDGVEVHNAKTKPREEQYNSTYRVVSVLTVLHQDWLNGKEYKCKVSNKALPAPIEKTISKAKGQPREPQVYTLPPSREEMTKNQVSLTCLVKGFYPSDIAVEWESNGQPENNYKTTPPVLDSDGSFFLYSKLTVDKSRWQQGNVFSCSVMHEALHNHYTQKSLSLSPG

SEQ ID NO: 12 - protein, 451 aa, synthetic construct
  REGION 1..451: note = Description of Artificial Sequence: Synthetic polypeptide
  VARIANT 1: note = /replace="pyro-Glu"
  SITE 1: note = MISC_FEATURE - /note="Variant residues given in the sequence have no preference with respect to those in the annotations for variant positions"
EVQLVQSGAEVEKPGASVKVSCKASGYTFASYGISWVRQAPGQGLEWMGGITPFFNRVDVAEKFQGRVTITADTSTNTVYIELSSLTSEDTAVYYCARDLRRGGVGDAFDIWGRGTLVTVSSASTKGPSVFPLAPSSKSTSGGTAALGCLVKDYFPEPVTVSWNSGALTSGVHTFPAVLQSSGLYSLSSVVTVPSSSLGTQTYICNVNHKPSNTKVDKRVEPKSCDKTHTCPPCPAPELLGGPSVFLFPPKPKDTLMISRTPEVTCVVVDVSHEDPEVKFNWYVDGVEVHNAKTKPREEQYASTYRVVSVLTVLHQDWLNGKEYKCKVSNKALPAPIEKTISKAKGQPREPQVYTLPPSREEMTKNQVSLTCLVKGFYPSDIAVEWESNGQPENNYKTTPPVLDSDGSFFLYSKLTVDKSRWQQGNVFSCSVMHEALHNHYTQKSLSLSPG

SEQ ID NO: 13 - protein, 451 aa, synthetic construct
  REGION 1..451: note = Description of Artificial Sequence: Synthetic polypeptide
  VARIANT 1: note = /replace="pyro-Glu"
  SITE 1: note = MISC_FEATURE - /note="Variant residues given in the sequence have no preference with respect to those in the annotations for variant positions"
EVQLVQSGAEVEKPGASVKVSCKASGYTFASYGISWVRQAPGQGLEWMGGITPFFNRVDVAEKFQGRVTITADTSTNTVYIELSSLTSEDTAVYYCARDLRRGGVGDAFDIWGRGTLVTVSSASTKGPSVFPLAPSSKSTSGGTAALGCLVKDYFPEPVTVSWNSGALTSGVHTFPAVLQSSGLYSLSSVVTVPSSSLGTQTYICNVNHKPSNTKVDKRVEPKSCDKTHTCPPCPAPEFFGGPSVFLFPPKPKDTLMISRTPEVTCVVVDVSHEDPEVKFNWYVDGVEVHNAKTKPREEQYASTYRVVSVLTVLHQDWLNGKEYKCKVSNKALPAPIEKTISKAKGQPREPQVYTLPPSREEMTKNQVSLTCLVKGFYPSDIAVEWESNGQPENNYKTTPPVLDSDGSFFLYSKLTVDKSRWQQGNVFSCSVMHEALHNHYTQKSLSLSPG

SEQ ID NO: 14 - protein, 451 aa, synthetic construct
  REGION 1..451: note = Description of Artificial Sequence: Synthetic polypeptide
  VARIANT 1: note = /replace="pyro-Glu"
  SITE 1: note = MISC_FEATURE - /note="Variant residues given in the sequence have no preference with respect to those in the annotations for variant positions"
EVQLVQSGAEVEKPGASVKVSCKASGYTFASYGISWVRQAPGQGLEWMGGITPFFNRVDVAEKFQGRVTITADTSTNTVYIELSSLTSEDTAVYYCARDLRRGGVGDAFDIWGRGTLVTVSSASTKGPSVFPLAPSSKSTSGGTAALGCLVKDYFPEPVTVSWNSGALTSGVHTFPAVLQSSGLYSLSSVVTVPSSSLGTQTYICNVNHKPSNTKVDKRVEPKSCDKTHTCPPCPAPELLGGPDVFLFPPKPKDTLMISRTPEVTCVVVDVSHEDPEVKFNWYVDGVEVHNAKTKPREEQYNSTYRVVSVLTVLHQDWLNGKEYKCKVSNKALPAPEEKTISKAKGQPREPQVYTLPPSREEMTKNQVSLTCLVKGFYPSDIAVEWESNGQPENNYKTTPPVLDSDGSFFLYSKLTVDKSRWQQGNVFSCSVMHEALHNHYTQKSLSLSPG

SEQ ID NO: 15 - protein, 451 aa, synthetic construct
  REGION 1..451: note = Description of Artificial Sequence: Synthetic polypeptide
  VARIANT 1: note = /replace="pyro-Glu"
  SITE 1: note = MISC_FEATURE - /note="Variant residues given in the sequence have no preference with respect to those in the annotations for variant positions"
EVQLVQSGAEVEKPGASVKVSCKASGYTFASYGISWVRQAPGQGLEWMGGITPFFNRVDVAEKFQGRVTITADTSTNTVYIELSSLTSEDTAVYYCARDLRRGGVGDAFDIWGRGTLVTVSSASTKGPSVFPLAPSSKSTSGGTAALGCLVKDYFPEPVTVSWNSGALTSGVHTFPAVLQSSGLYSLSSVVTVPSSSLGTQTYICNVNHKPSNTKVDKRVEPKSCDKTHTCPPCPAPELLGGPDVFLFPPKPKDTLMISRTPEVTCVVVDVSHEDPEVKFNWYVDGVEVHNAKTKPREEQYNSTYRVVSVLTVLHQDWLNGKEYKCKVSNKALPLPEEKTISKAKGQPREPQVYTLPPSREEMTKNQVSLTCLVKGFYPSDIAVEWESNGQPENNYKTTPPVLDSDGSFFLYSKLTVDKSRWQQGNVFSCSVMHEALHNHYTQKSLSLSPG

SEQ ID NO: 16 - protein, 451 aa, synthetic construct
  REGION 1..451: note = Description of Artificial Sequence: Synthetic polypeptide
  VARIANT 1: note = /replace="pyro-Glu"
  SITE 1: note = MISC_FEATURE - /note="Variant residues given in the sequence have no preference with respect to those in the annotations for variant positions"
EVQLVQSGAEVEKPGASVKVSCKASGYTFASYGISWVRQAPGQGLEWMGGITPFFNRVDVAEKFQGRVTITADTSTNTVYIELSSLTSEDTAVYYCARDLRRGGVGDAFDIWGRGTLVTVSSASTKGPSVFPLAPSSKSTSGGTAALGCLVKDYFPEPVTVSWNSGALTSGVHTFPAVLQSSGLYSLSSVVTVPSSSLGTQTYICNVNHKPSNTKVDKRVEPKSCDKTHTCPPCPAPELVGGPSVFLLPPKPKDTLMISRTPEVTCVVVDVSHEDPEVKFNWYVDGVEVHNAKTKPPEEQYNSTLRVVSVLTVLHQDWLNGKEYKCKVSNKALPAPIEKTISKAKGQPREPQVYTLPPSREEMTKNQVSLTCLVKGFYPSDIAVEWESNGQPENNYKTTPLVLDSDGSFFLYSKLTVDKSRWQQGNVFSCSVMHEALHNHYTQKSLSLSPG

SEQ ID NO: 17 - protein, 451 aa, synthetic construct
  REGION 1..451: note = Description of Artificial Sequence: Synthetic polypeptide
  VARIANT 1: note = /replace="pyro-Glu"
  SITE 1: note = MISC_FEATURE - /note="Variant residues given in the sequence have no preference with respect to those in the annotations for variant positions"
EVQLVQSGAEVEKPGASVKVSCKASGYTFASYGISWVRQAPGQGLEWMGGITPFFNRVDVAEKFQGRVTITADTSTNTVYIELSSLTSEDTAVYYCARDLRRGGVGDAFDIWGRGTLVTVSSASTKGPSVFPLAPSSKSTSGGTAALGCLVKDYFPEPVTVSWNSGALTSGVHTFPAVLQSSGLYSLSSVVTVPSSSLGTQTYICNVNHKPSNTKVDKRVEPKSCDKTHTCPPCPAPELLGGPSVFLFPPKPKDTLMISRTPEVTCVVVDVEHEDPEVKFNWYVDGVEVHNAKTKPREEQYNSTYRVVSVLTVLHQDWLNGKEYKCKVSNKAFPAPIEKTISKAKGQPREPQVYTLPPSREEMTKNQVSLTCLVKGFYPSDIAVEWESNGQPENNYKTTPPVLDSDGSFFLYSKLTVDKSRWQQGNVFSCSVMHEALHNHYTQKSLSLSPG

SEQ ID NO: 18 - protein, 448 aa, synthetic construct
  REGION 1..448: note = Description of Artificial Sequence: Synthetic polypeptide
  VARIANT 1: note = /replace="pyro-Glu"
  SITE 1: note = MISC_FEATURE - /note="Variant residues given in the sequence have no preference with respect to those in the annotations for variant positions"
EVQLVQSGAEVEKPGASVKVSCKASGYTFASYGISWVRQAPGQGLEWMGGITPFFNRVDVAEKFQGRVTITADTSTNTVYIELSSLTSEDTAVYYCARDLRRGGVGDAFDIWGRGTLVTVSSASTKGPSVFPLAPCSRSTSESTAALGCLVKDYFPEPVTVSWNSGALTSGVHTFPAVLQSSGLYSLSSVVTVPSSSLGTKTYTCNVDHKPSNTKVDKRVESKYGPPCPPCPAPEFLGGPSVFLFPPKPKDTLMISRTPEVTCVVVDVSQEDPEVQFNWYVDGVEVHNAKTKPREEQFNSTYRVVSVLTVLHQDWLNGKEYKCKVSNKGLPSSIEKTISKAKGQPREPQVYTLPPSQEEMTKNQVSLTCLVKGFYPSDIAVEWESNGQPENNYKTTPPVLDSDGSFFLYSRLTVDKSRWQEGNVFSCSVMHEALHNHYTQKSLSLSLG

SEQ ID NO: 19 - protein, 329 aa, synthetic construct
  REGION 1..329: note = Description of Artificial Sequence: Synthetic polypeptide
ASTKGPSVFPLAPSSKSTSGGTAALGCLVKDYFPEPVTVSWNSGALTSGVHTFPAVLQSSGLYSLSSVVTVPSSSLGTQTYICNVNHKPSNTKVDKRVEPKSCDKTHTCPPCPAPELLGGPSVFLFPPKPKDTLMISRTPEVTCVVVDVSHEDPEVKFNWYVDGVEVHNAKTKPREEQYNSTYRVVSVLTVLHQDWLNGKEYKCKVSNKALPAPIEKTISKAKGQPREPQVYTLPPSREEMTKNQVSLTCLVKGFYPSDIAVEWESNGQPENNYKTTPPVLDSDGSFFLYSKLTVDKSRWQQGNVFSCSVMHEALHNHYTQKSLSLSPG

SEQ ID NO: 20 - protein, 329 aa, synthetic construct
  REGION 1..329: note = Description of Artificial Sequence: Synthetic polypeptide
ASTKGPSVFPLAPSSKSTSGGTAALGCLVKDYFPEPVTVSWNSGALTSGVHTFPAVLQSSGLYSLSSVVTVPSSSLGTQTYICNVNHKPSNTKVDKRVEPKSCDKTHTCPPCPAPELLGGPSVFLFPPKPKDTLMISRTPEVTCVVVDVSHEDPEVKFNWYVDGVEVHNAKTKPREEQYASTYRVVSVLTVLHQDWLNGKEYKCKVSNKALPAPIEKTISKAKGQPREPQVYTLPPSREEMTKNQVSLTCLVKGFYPSDIAVEWESNGQPENNYKTTPPVLDSDGSFFLYSKLTVDKSRWQQGNVFSCSVMHEALHNHYTQKSLSLSPG

SEQ ID NO: 21 - protein, 329 aa, synthetic construct
  REGION 1..329: note = Description of Artificial Sequence: Synthetic polypeptide
ASTKGPSVFPLAPSSKSTSGGTAALGCLVKDYFPEPVTVSWNSGALTSGVHTFPAVLQSSGLYSLSSVVTVPSSSLGTQTYICNVNHKPSNTKVDKRVEPKSCDKTHTCPPCPAPEFFGGPSVFLFPPKPKDTLMISRTPEVTCVVVDVSHEDPEVKFNWYVDGVEVHNAKTKPREEQYASTYRVVSVLTVLHQDWLNGKEYKCKVSNKALPAPIEKTISKAKGQPREPQVYTLPPSREEMTKNQVSLTCLVKGFYPSDIAVEWESNGQPENNYKTTPPVLDSDGSFFLYSKLTVDKSRWQQGNVFSCSVMHEALHNHYTQKSLSLSPG

SEQ ID NO: 22 - protein, 329 aa, synthetic construct
  REGION 1..329: note = Description of Artificial Sequence: Synthetic polypeptide
ASTKGPSVFPLAPSSKSTSGGTAALGCLVKDYFPEPVTVSWNSGALTSGVHTFPAVLQSSGLYSLSSVVTVPSSSLGTQTYICNVNHKPSNTKVDKRVEPKSCDKTHTCPPCPAPELLGGPDVFLFPPKPKDTLMISRTPEVTCVVVDVSHEDPEVKFNWYVDGVEVHNAKTKPREEQYNSTYRVVSVLTVLHQDWLNGKEYKCKVSNKALPAPEEKTISKAKGQPREPQVYTLPPSREEMTKNQVSLTCLVKGFYPSDIAVEWESNGQPENNYKTTPPVLDSDGSFFLYSKLTVDKSRWQQGNVFSCSVMHEALHNHYTQKSLSLSPG

SEQ ID NO: 23 - protein, 329 aa, synthetic construct
  REGION 1..329: note = Description of Artificial Sequence: Synthetic polypeptide
ASTKGPSVFPLAPSSKSTSGGTAALGCLVKDYFPEPVTVSWNSGALTSGVHTFPAVLQSSGLYSLSSVVTVPSSSLGTQTYICNVNHKPSNTKVDKRVEPKSCDKTHTCPPCPAPELLGGPDVFLFPPKPKDTLMISRTPEVTCVVVDVSHEDPEVKFNWYVDGVEVHNAKTKPREEQYNSTYRVVSVLTVLHQDWLNGKEYKCKVSNKALPLPEEKTISKAKGQPREPQVYTLPPSREEMTKNQVSLTCLVKGFYPSDIAVEWESNGQPENNYKTTPPVLDSDGSFFLYSKLTVDKSRWQQGNVFSCSVMHEALHNHYTQKSLSLSPG

SEQ ID NO: 24 - protein, 329 aa, synthetic construct
  REGION 1..329: note = Description of Artificial Sequence: Synthetic polypeptide
ASTKGPSVFPLAPSSKSTSGGTAALGCLVKDYFPEPVTVSWNSGALTSGVHTFPAVLQSSGLYSLSSVVTVPSSSLGTQTYICNVNHKPSNTKVDKRVEPKSCDKTHTCPPCPAPELVGGPSVFLLPPKPKDTLMISRTPEVTCVVVDVSHEDPEVKFNWYVDGVEVHNAKTKPPEEQYNSTLRVVSVLTVLHQDWLNGKEYKCKVSNKALPAPIEKTISKAKGQPREPQVYTLPPSREEMTKNQVSLTCLVKGFYPSDIAVEWESNGQPENNYKTTPLVLDSDGSFFLYSKLTVDKSRWQQGNVFSCSVMHEALHNHYTQKSLSLSPG

SEQ ID NO: 25 - protein, 329 aa, synthetic construct
  REGION 1..329: note = Description of Artificial Sequence: Synthetic polypeptide
ASTKGPSVFPLAPSSKSTSGGTAALGCLVKDYFPEPVTVSWNSGALTSGVHTFPAVLQSSGLYSLSSVVTVPSSSLGTQTYICNVNHKPSNTKVDKRVEPKSCDKTHTCPPCPAPELLGGPSVFLFPPKPKDTLMISRTPEVTCVVVDVEHEDPEVKFNWYVDGVEVHNAKTKPREEQYNSTYRVVSVLTVLHQDWLNGKEYKCKVSNKAFPAPIEKTISKAKGQPREPQVYTLPPSREEMTKNQVSLTCLVKGFYPSDIAVEWESNGQPENNYKTTPPVLDSDGSFFLYSKLTVDKSRWQQGNVFSCSVMHEALHNHYTQKSLSLSPG

SEQ ID NO: 26 - protein, 326 aa, synthetic construct
  REGION 1..326: note = Description of Artificial Sequence: Synthetic polypeptide
ASTKGPSVFPLAPCSRSTSESTAALGCLVKDYFPEPVTVSWNSGALTSGVHTFPAVLQSSGLYSLSSVVTVPSSSLGTKTYTCNVDHKPSNTKVDKRVESKYGPPCPPCPAPEFLGGPSVFLFPPKPKDTLMISRTPEVTCVVVDVSQEDPEVQFNWYVDGVEVHNAKTKPREEQFNSTYRVVSVLTVLHQDWLNGKEYKCKVSNKGLPSSIEKTISKAKGQPREPQVYTLPPSQEEMTKNQVSLTCLVKGFYPSDIAVEWESNGQPENNYKTTPPVLDSDGSFFLYSRLTVDKSRWQEGNVFSCSVMHEALHNHYTQKSLSLSLG

SEQ ID NO: 27 - protein, 216 aa, synthetic construct
  REGION 1..216: note = Description of Artificial Sequence: Synthetic polypeptide
  VARIANT 1: note = /replace="pyro-Glu"
  SITE 1: note = MISC_FEATURE - /note="Variant residues given in the sequence have no preference with respect to those in the annotations for variant positions"
ESALTQPRSVSGSPGQSVTISCTGTSSDVGSHNYVSWYQQHPGKAPQLMIYEVSYRPSEISNRFSGSKSGNTASLTISGLQPEDEADYYCSSYTPSSATVFGAGTKLTVLGQPKAAPSVTLFPPSSEELQANKATLVCLISDFYPGAVTVAWKADSSPVKAGVETTTPSKQSNNKYAASSYLSLTPEQWKSHRSYSCQVTHEGSTVEKTVAPTECS

SEQ ID NO: 28 - protein, 106 aa, synthetic construct
  REGION 1..106: note = Description of Artificial Sequence: Synthetic polypeptide
GQPKAAPSVTLFPPSSEELQANKATLVCLISDFYPGAVTVAWKADSSPVKAGVETTTPSKQSNNKYAASSYLSLTPEQWKSHRSYSCQVTHEGSTVEKTVAPTECS

SEQ ID NO: 29 - protein, 244 aa, Homo sapiens
MRWCLLLIWAQGLRQAPLASGMMTGTIETTGNISAEKGGSIILQCHLSSTTAQVTQVNWEQQDQLLAICNADLGWHISPSFKDRVAPGPGLGLTLQSLTVNDTGEYFCIYHTYPDGTYTGRIFLEVLESSVAEHGARFQIPLLGAMAATLVVICTAVIVVVALTRKKKALRIHSVEGDLRRKSAGQEEWSPSAPSPPGSCVQAEAAPAGLCGEQRGEDCAELHDYFNVLSYRSLGNCSFFTETG

SEQ ID NO: 30 - protein, 117 aa, synthetic construct
  REGION 1..117: note = Description of Artificial Sequence: Synthetic polypeptide
MMTGTIETTGNISAEKGGSIILQCHLSSTTAQVTQVNWEQQDQLLAICNADLGWHISPSFKDRVAPGPGLGLTLQSLTVNDTGEYFCIYHTYPDGTYTGRIFLEVLESSVAEHGARF

SEQ ID NO: 31 - protein, 16 aa, synthetic construct
  REGION 1..16: note = Description of Artificial Sequence: Synthetic peptide
YHTYPDGTYTGRIFLE

SEQ ID NO: 32 - protein, 4 aa, synthetic construct
  REGION 1..4: note = Description of Artificial Sequence: Synthetic peptide
VTQV

SEQ ID NO: 33 - protein, 14 aa, synthetic construct
  REGION 1..14: note = Description of Artificial Sequence: Synthetic peptide
ICNADLGWHISPSF

SEQ ID NO: 34 - protein, 98 aa, synthetic construct
  REGION 1..98: note = Description of Artificial Sequence: Synthetic polypeptide
QVQLVQSGAEVKKPGSSVKVSCKASGGTFSSYAISWVRQAPGQGLEWMGGIIPIFGTANYAQKFQGRVTITADESTSTAYMELSSLRSEDTAVYYCAR

SEQ ID NO: 35 - protein, 98 aa, synthetic construct
  REGION 1..98: note = Description of Artificial Sequence: Synthetic polypeptide
QVQLVQSGAEVKKPGSSVKVSCKASGGTFSSYAISWVRQAPGQGLEWMGGIIPIFGTANYAQKFQGRVTITADKSTSTAYMELSSLRSEDTAVYYCAR

SEQ ID NO: 36 - protein, 118 aa, synthetic construct
  REGION 1..118: note = Description of Artificial Sequence: Synthetic polypeptide
MMTGTIETTGNISAEKGGSIILQCHLSSTTAQVTQVNWEQQDQLLAICSADLGWHISPSFKDRVAPGPGLGLTLQSLTVNDTGEYFCIYHTYPDGTYTGRIFLEVLESSVAEHGARFQ

SEQ ID NO: 37 - protein, 99 aa, synthetic construct
  REGION 1..99: note = Description of Artificial Sequence: Synthetic polypeptide
QSALTQPASVSGSPGQSITISCTGTSSDVGGYNYVSWYQQHPGKAPKLMIYEVSNRPSGVSNRFSGSKSGNTASLTISGLQAEDEADYYCSSYTSSSTL

SEQ ID NO: 38 - protein, 99 aa, synthetic construct
  REGION 1..99: note = Description of Artificial Sequence: Synthetic polypeptide
QSALTQPASVSGSPGQSITISCTGTSSDVGSYNLVSWYQQHPGKAPKLMIYEVSKRPSGVSNRFSGSKSGNTASLTISGLQAEDEADYYCCSYAGSSTF

SEQ ID NO: 39 - protein, 99 aa, synthetic construct
  REGION 1..99: note = Description of Artificial Sequence: Synthetic polypeptide
QSALTQPRSVSGSPGQSVTISCTGTSSDVGGYNYVSWYQQHPGKAPKLMIYDVSKRPSGVPDRFSGSKSGNTASLTISGLQAEDEADYYCCSYAGSYTF

SEQ ID NO: 40 - protein, 223 aa, synthetic construct [sequence omitted]

SEQ ID NO: 41 - protein, 120 aa, synthetic construct
  REGION 1..120: note = Description of Artificial Sequence: Synthetic polypeptide
MMTGTIETTGNISAEKGGSIILQCHLSSTTAQVTQVNWEQQDQLLAICNADLGWHISPSFKDRVAPGPGLGLTLQSLTVNDTGEYFCIYHTYPDGTYTGRIFLEVLESSVAEHGARFQIP

SEQ ID NO: 42 - protein, 118 aa, synthetic construct
  REGION 1..118: note = Description of Artificial Sequence: Synthetic polypeptide
MMTGTIETTGNISAEKGGSIILQCHLSSTTAQVTQVNWEQQDQLLAICNADLGWHISPSFKDRVAPGPGLGLTLQSLTVNDTGEYFCIYHTYPDGTYTGRIFLEVLESSVAEHGARFQ

SEQ ID NO: 43 - protein, 118 aa, synthetic construct
  REGION 1..118: note = Description of Artificial Sequence: Synthetic polypeptide
MMTGTIETTGNISAEKGGSIILQCHLSSTTAQVAQVNWEQQDQLLAICNADLGWHISPSFKDRVAPGPGLGLTLQSLTVNDTGEYFCIYHTYPDGTYTGRIFLEVLESSVAEHGARFQ

SEQ ID NO: 44 - protein, 118 aa, synthetic construct
  REGION 1..118: note = Description of Artificial Sequence: Synthetic polypeptide
MMTGTIETTGNISAEKGGSIILQCHLSSTTAQVTAVNWEQQDQLLAICNADLGWHISPSFKDRVAPGPGLGLTLQSLTVNDTGEYFCIYHTYPDGTYTGRIFLEVLESSVAEHGARFQ

SEQ ID NO: 45 - protein, 118 aa, synthetic construct
  REGION 1..118: note = Description of Artificial Sequence: Synthetic polypeptide
MMTGTIETTGNISAEKGGSIILQCHLSSTTAQVTQVNWEQQDQLLAECNADLGWHISPSFKDRVAPGPGLGLTLQSLTVNDTGEYFCIYHTYPDGTYTGRIFLEVLESSVAEHGARFQ

SEQ ID NO: 46 - protein, 118 aa, synthetic construct
  REGION 1..118: note = Description of Artificial Sequence: Synthetic polypeptide
MMTGTIETTGNISAEKGGSIILQCHLSSTTAQVTQVNWEQQDQLLAICAADLGWHISPSFKDRVAPGPGLGLTLQSLTVNDTGEYFCIYHTYPDGTYTGRIFLEVLESSVAEHGARFQ

SEQ ID NO: 47 - protein, 118 aa, synthetic construct
  REGION 1..118: note = Description of Artificial Sequence: Synthetic polypeptide
MMTGTIETTGNISAEKGGSIILQCHLSSTTAQVTQVNWEQQDQLLAICNADAGWHISPSFKDRVAPGPGLGLTLQSLTVNDTGEYFCIYHTYPDGTYTGRIFLEVLESSVAEHGARFQ

SEQ ID NO: 48 - protein, 118 aa, synthetic construct
  REGION 1..118: note = Description of Artificial Sequence: Synthetic polypeptide
MMTGTIETTGNISAEKGGSIILQCHLSSTTAQVTQVNWEQQDQLLAICNADEGWHISPSFKDRVAPGPGLGLTLQSLTVNDTGEYFCIYHTYPDGTYTGRIFLEVLESSVAEHGARFQ

SEQ ID NO: 49 - protein, 118 aa, synthetic construct
  REGION 1..118: note = Description of Artificial Sequence: Synthetic polypeptide
MMTGTIETTGNISAEKGGSIILQCHLSSTTAQVTQVNWEQQDQLLAICNADLGWAISPSFKDRVAPGPGLGLTLQSLTVNDTGEYFCIYHTYPDGTYTGRIFLEVLESSVAEHGARFQ

SEQ ID NO: 50 - protein, 118 aa, synthetic construct
  REGION 1..118: note = Description of Artificial Sequence: Synthetic polypeptide
MMTGTIETTGNISAEKGGSIILQCHLSSTTAQVTQVNWEQQDQLLAICNADLGWHISASFKDRVAPGPGLGLTLQSLTVNDTGEYFCIYHTYPDGTYTGRIFLEVLESSVAEHGARFQ

SEQ ID NO: 51 - protein, 118 aa, synthetic construct
  REGION 1..118: note = Description of Artificial Sequence: Synthetic polypeptide
MMTGTIETTGNISAEKGGSIILQCHLSSTTAQVTQVNWEQQDQLLAICNADLGWHISPSFKDRVAPGPGLGLTLQSLTVNDTGEYFCIYATYPDGTYTGRIFLEVLESSVAEHGARFQ

SEQ ID NO: 52 - protein, 118 aa, synthetic construct
  REGION 1..118: note = Description of Artificial Sequence: Synthetic polypeptide
MMTGTIETTGNISAEKGGSIILQCHLSSTTAQVTQVNWEQQDQLLAICNADLGWHISPSFKDRVAPGPGLGLTLQSLTVNDTGEYFCIYHTYPDGAYTGRIFLEVLESSVAEHGARFQ

SEQ ID NO: 53 - protein, 118 aa, synthetic construct
  REGION 1..118: note = Description of Artificial Sequence: Synthetic polypeptide
MMTGTIETTGNISAEKGGSIILQCHLSSTTAQVTQVNWEQQDQLLAICNADLGWHISPSFKDRVAPGPGLGLTLQSLTVNDTGEYFCIYHTYPDGIYTGRIFLEVLESSVAEHGARFQ

SEQ ID NO: 54 - protein, 118 aa, synthetic construct
  REGION 1..118: note = Description of Artificial Sequence: Synthetic polypeptide
MMTGTIETTGNISAEKGGSIILQCHLSSTTAQVTQVNWEQQDQLLAICNADLGWHISPSFKDRVAPGPGLGLTLQSLTVNDTGEYFCIYHTYPDGTYAGRIFLEVLESSVAEHGARFQ

SEQ ID NO: 55 - protein, 118 aa, synthetic construct
  REGION 1..118: note = Description of Artificial Sequence: Synthetic polypeptide
MMTGTIETTGNISAEKGGSIILQCHLSSTTAQVTQVNWEQQDQLLAICNADLGWHISPSFKDRVAPGPGLGLTLQSLTVNDTGEYFCIYHTYPDGTYTGAIFLEVLESSVAEHGARFQ

SEQ ID NO: 56 - protein, 118 aa, synthetic construct
  REGION 1..118: note = Description of Artificial Sequence: Synthetic polypeptide
MMTGTIETTGNISAEKGGSIILQCHLSSTTAQVTQVNWEQQDQLLAICNADLGWHISPSFKDRVAPGPGLGLTLQSLTVNDTGEYFCIYHTYPDGTYTGRIALEVLESSVAEHGARFQ

SEQ ID NO: 57 - protein, 118 aa, synthetic construct
  REGION 1..118: note = Description of Artificial Sequence: Synthetic polypeptide
MMTGTIETTGNISAEKGGSIILQCHLSSTTAQVTQVNWEQQDQLLAIYSVDLGWHISPSFKDRVAPGPGLGLTLQSLTVNDTGEYFCIYHTYPDGTYTGRIFLEVLESSVAEHGARFQ

SEQ ID NO: 58 - protein, 118 aa, synthetic construct
  REGION 1..118: note = Description of Artificial Sequence: Synthetic polypeptide
MMTGTIETTGNISAEKGGSIILQCHLSSTTAQVTQVNWEQQDQLLAICNADLGWHVASVFKDRVAPGPGLGLTLQSLTVNDTGEYFCIYHTYPDGTYTGRIFLEVLESSVAEHGARFQ

SEQ ID NO: 59 - protein, 118 aa, synthetic construct
  REGION 1..118: note = Description of Artificial Sequence: Synthetic polypeptide
MMTGTIETTGNISAEKGGSIILQCHLSSTTAQVTQVNWEQQDQLLAICNADLGWHISPSFKDRVAPGPGLGLTLQSLTVNDTGEYFCIYHTYPDGIYKGRIFLEVLESSVAEHGARFQ

SEQ ID NO: 60 - protein, 99 aa, synthetic construct
  REGION 1..99: note = Description of Artificial Sequence: Synthetic polypeptide
QSALTQPASVSGSPGQSITISCTGTSSDVGSYNLVSWYQQHPGKAPKLMIYEGSKRPSGVSNRFSGSKSGNTASLTISGLQAEDEADYYCSSYTSSSTL

SEQ ID NO: 61 - protein, 9 aa, unidentified
NLVPMVATV

SEQ ID NO: 62 - protein, 119 aa, synthetic construct
  REGION 1..119: note = Description of Artificial Sequence: Synthetic polypeptide
  VARIANT 1: note = /replace="pyro-Glu"
  SITE 1: note = MISC_FEATURE - /note="Variant residues given in the sequence have no preference with respect to those in the annotations for variant positions"
EVQLVESGGGLTQPGKSLKLSCEASGFTFSSFTMHWVRQSPGKGLEWVAFIRSGSGIVFYADAVRGRFTISRDNAKNLLFLQMNDLKSEDTAMYYCARRPLGHNTFDSWGQGTLVTVSS

SEQ ID NO: 63 - protein, 113 aa, synthetic construct
  REGION 1..113: note = Description of Artificial Sequence: Synthetic polypeptide
DIVMTQSPSSLAVSPGEKVTMTCKSSQSLYYSGVKENLLAWYQQKPGQSPKLLIYYASIRFTGVPDRFTGSGSGTDYTLTITSVQAEDMGQYFCQQGINNPLTFGDGTKLEIK

SEQ ID NO: 64 - protein, 448 aa, synthetic construct
  REGION 1..448: note = Description of Artificial Sequence: Synthetic polypeptide
  VARIANT 1: note = /replace="pyro-Glu"
  SITE 1: note = MISC_FEATURE - /note="Variant residues given in the sequence have no preference with respect to those in the annotations for variant positions"
EVQLVESGGGLTQPGKSLKLSCEASGFTFSSFTMHWVRQSPGKGLEWVAFIRSGSGIVFYADAVRGRFTISRDNAKNLLFLQMNDLKSEDTAMYYCARRPLGHNTFDSWGQGTLVTVSSAKTTAPSVYPLAPVCGDTTGSSVTLGCLVKGYFPEPVTLTWNSGSLSSGVHTFPAVLQSDLYTLSSSVTVTSSTWPSQSITCNVAHPASSTKVDKKIEPRGPTIKPCPPCKCPAPNLLGGPSVFIFPPKIKDVLMISLSPIVTCVVVDVSEDDPDVQISWFVNNVEVHTAQTQTHREDYNSTLRVVSALPIQHQDWMSGKEFKCKVNNKDLPAPIERTISKPKGSVRAPQVYVLPPPEEEMTKKQVTLTCMVTDFMPEDIYVEWTNNGKTELNYKNTEPVLDSDGSYFMYSKLRVEKKNWVERNSYSCSVVHEGLHNHHTTKSFSRTPG

SEQ ID NO: 65 - protein, 449 aa, synthetic construct
  REGION 1..449: note = Description of Artificial Sequence: Synthetic polypeptide
  VARIANT 1: note = /replace="pyro-Glu"
  SITE 1: note = MISC_FEATURE - /note="Variant residues given in the sequence have no preference with respect to those in the annotations for variant positions"
EVQLVESGGGLTQPGKSLKLSCEASGFTFSSFTMHWVRQSPGKGLEWVAFIRSGSGIVFYADAVRGRFTISRDNAKNLLFLQMNDLKSEDTAMYYCARRPLGHNTFDSWGQGTLVTVSSAKTTAPSVYPLAPVCGDTTGSSVTLGCLVKGYFPEPVTLTWNSGSLSSGVHTFPAVLQSDLYTLSSSVTVTSSTWPSQSITCNVAHPASSTKVDKKIEPRGPTIKPCPPCKCPAPNLLGGPSVFIFPPKIKDVLMISLSPIVTCVVVDVSEDDPDVQISWFVNNVEVHTAQTQTHREDYNSTLRVVSALPIQHQDWMSGKEFKCKVNNKDLPAPIERTISKPKGSVRAPQVYVLPPPEEEMTKKQVTLTCMVTDFMPEDIYVEWTNNGKTELNYKNTEPVLDSDGSYFMYSKLRVEKKNWVERNSYSCSVVHEGLHNHHTTKSFSRTPGK

SEQ ID NO: 66 - protein, 449 aa, synthetic construct
  REGION 1..449: note = Description of Artificial Sequence: Synthetic polypeptide
  VARIANT 1: note = /replace="pyro-Glu"
  SITE 1: note = MISC_FEATURE - /note="Variant residues given in the sequence have no preference with respect to those in the annotations for variant positions"
EVQLVESGGGLTQPGKSLKLSCEASGFTFSSFTMHWVRQSPGKGLEWVAFIRSGSGIVFYADAVRGRFTISRDNAKNLLFLQMNDLKSEDTAMYYCARRPLGHNTFDSWGQGTLVTVSSAKTTAPSVYPLAPVCGDTTGSSVTLGCLVKGYFPEPVTLTWNSGSLSSGVHTFPAVLQSDLYTLSSSVTVTSSTWPSQSITCNVAHPASSTKVDKKIEPRGPTIKPCPPCKCPAPNLLGGPSVFIFPPKIKDVLMISLSPIVTCVVVDVSEDDPDVQISWFVNNVEVHTAQTQTHREDYQSTLRVVSALPIQHQDWMSGKEFKCKVNNKDLPAPIERTISKPKGSVRAPQVYVLPPPEEEMTKKQVTLTCMVTDFMPEDIYVEWTNNGKTELNYKNTEPVLDSDGSYFMYSKLRVEKKNWVERNSYSCSVVHEGLHNHHTTKSFSRTPGK

SEQ ID NO: 67 - protein, 443 aa, synthetic construct
  REGION 1..443: note = Description of Artificial Sequence: Synthetic polypeptide
  VARIANT 1: note = /replace="pyro-Glu"
  SITE 1: note = MISC_FEATURE - /note="Variant residues given in the sequence have no preference with respect to those in the annotations for variant positions"
EVQLVESGGGLTQPGKSLKLSCEASGFTFSSFTMHWVRQSPGKGLEWVAFIRSGSGIVFYADAVRGRFTISRDNAKNLLFLQMNDLKSEDTAMYYCARRPLGHNTFDSWGQGTLVTVSSAKTTPPSVYPLAPGSAAQTNSMVTLGCLVKGYFPEPVTVTWNSGSLSSGVHTFPAVLQSDLYTLSSSVTVPSSTWPSETVTCNVAHPASSTKVDKKIVPRDCGCKPCICTVPEVSSVFIFPPKPKDVLTITLTPKVTCVVVDISKDDPEVQFSWFVDDVEVHTAQTQPREEQFNSTFRSVSELPIMHQDWLNGKEFKCRVNSAAFPAPIEKTISKTKGRPKAPQVYTIPPPKEQMAKDKVSLTCMITDFFPEDITVEWQWNGQPAENYKNTQPIMDTDGSYFVYSKLNVQKSNWEAGNTFTCSVLHEGLHNHHTEKSLSHSPGK

SEQ ID NO: 68 - protein, 448 aa, synthetic construct
  REGION 1..448: note = Description of Artificial Sequence: Synthetic polypeptide
  VARIANT 1: note = /replace="pyro-Glu"
  SITE 1: note = MISC_FEATURE - /note="Variant residues given in the sequence have no preference with respect to those in the annotations for variant positions"
EVQLVESGGGLTQPGKSLKLSCEASGFTFSSFTMHWVRQSPGKGLEWVAFIRSGSGIVFYADAVRGRFTISRDNAKNLLFLQMNDLKSEDTAMYYCARRPLGHNTFDSWGQGTLVTVSSAKTTAPSVYPLAPVCGDTTGSSVTLGCLVKGYFPEPVTLTWNSGSLSSGVHTFPAVLQSDLYTLSSSVTVTSSTWPSQSITCNVAHPASSTKVDKKIEPRGPTIKPCPPCKCPAPNLLGGPDVFIFPPKIKDVLMISLSPIVTCVVVDVSEDDPDVQISWFVNNVEVHTAQTQTHREDYNSTLRVVSALPIQHQDWMSGKEFKCKVNNKDLPLPEERTISKPKGSVRAPQVYVLPPPEEEMTKKQVTLTCMVTDFMPEDIYVEWTNNGKTELNYKNTEPVLDSDGSYFMYSKLRVEKKNWVERNSYSCSVVHEGLHNHHTTKSFSRTPG

SEQ ID NO: 69 - protein, 220 aa, synthetic construct
  REGION 1..220: note = Description of Artificial Sequence: Synthetic polypeptide
DIVMTQSPSSLAVSPGEKVTMTCKSSQSLYYSGVKENLLAWYQQKPGQSPKLLIYYASIRFTGVPDRFTGSGSGTDYTLTITSVQAEDMGQYFCQQGINNPLTFGDGTKLEIKRADAAPTVSIFPPSSEQLTSGGASVVCFLNNFYPKDINVKWKIDGSERQNGVLNSWTDQDSKDSTYSMSSTLTLTKDEYERHNSYTCEATHKTSTSPIVKSFNRNEC

SEQ ID NO: 70 - protein, 245 aa, Macaca fascicularis
MRWCLFLIWAQGLRQAPLASGMMTGTIETTGNISAKKGGSVILQCHLSSTMAQVTQVNWEQHDHSLLAIRNAELGWHIYPAFKDRVAPGPGLGLTLQSLTMNDTGEYFCTYHTYPDGTYRGRIFLEVLESSVAEHSARFQIPLLGAMAMMLVVICIAVIVVVVLARKKKSLRIHSVESGLQRKSTGQEEQIPSAPSPPGSCVQAEAAPAGLCGEQQGDDCAELHDYFNVLSYRSLGSCSFFTETG